European Patent Application EP 4 282 423 A1, published November 29, 2023. Title: PHARMACEUTICAL COMPOSITION COMPRISING MESENCHYMAL STEM CELLS EXPRESSING PTX-3, TIMP1 AND BDNF AS EFFECTIVE INGREDIENTS FOR PREVENTION OR TREATMENT OF INFLAMMATORY DISEASE OR PAIN. Applicant: MEDIPOST CO., LTD. The sequence listing filed with the application follows.

SEQUENCE LISTING (8 sequences)

SEQ ID NO: 1 - DNA, 19 bp, Artificial Sequence
  nucleotide sequence for primer_Human GAPDH(forward)
agccacatcgctcagacac

SEQ ID NO: 2 - DNA, 19 bp, Artificial Sequence
  nucleotide sequence for primer_Human GAPDH(reverse)
gcccaatacgaccaaatcc

SEQ ID NO: 3 - DNA, 20 bp, Artificial Sequence
  nucleotide sequence for primer_Human IL-1b(forward)
tacctgtcctgcgtcttgaa

SEQ ID NO: 4 - DNA, 23 bp, Artificial Sequence
  nucleotide sequence for primer_Human IL-1b(reverse)
tctttgggtaatttttgggatct

SEQ ID NO: 5 - DNA, 20 bp, Artificial Sequence
  nucleotide sequence for primer_Human IL-8(forward)
agacagcagagcacacaagc

SEQ ID NO: 6 - DNA, 18 bp, Artificial Sequence
  nucleotide sequence for primer_Human IL-8(reverse)
atggttccttccggtggt

SEQ ID NO: 7 - DNA, 24 bp, Artificial Sequence
  nucleotide sequence for primer_Human IL-6(forward)
gatgagtacaaaagtcctgatcca

SEQ ID NO: 8 - DNA, 19 bp, Artificial Sequence
  nucleotide sequence for primer_Human IL-6(reverse)
ctgcagccactggttctgt